European Patent Specification EP 4 087 879 B1, published May 6, 2026. Title: Anti MUC1-SEA antibodies. Applicant: BioModifying, LLC. The sequence listing filed with the application follows.

SEQUENCE LISTING (60 sequences)

SEQ ID NO: 1 - DNA, 420 bp, Mus musculus
atgagagtgctgattcttttgtgcctgttcacagcctttcctggtgtcctgtctgatgtgcaggttcaggagtcaggacctgacctggtgaaaccttctcagtcactttctctcacctgcactgtcactggccactccatcaccagaggttctagctggcactggatccggcagtttccaggaaacaaactggagtggatgggatacatacattacggtggtggcacttcctacaacccatctctcaaaagtcgaatctctatcactcgagacacatccaagaaccagttcttcctgcagttgaattctgtgactactgaggacacagccacatttttctgtgcacggtattcctacgatattacctaccgctggttcttcgatgtctggggcgcagggaccacggtcatcgtctcctca

SEQ ID NO: 2 - DNA, 381 bp, mus Musculus
atggtatccacacctcagttccttgtatttttgcttttctggattccagcctccagaggtgacatcttgctgactcagtctccagccatcctgtctgtgagtccaggagaaagagtcagtttctcctgcagggccagtcagaacattggcacaagcatacactggtatcagcaaagaaaaaatggttctccaagacttctcataaagtatgcttctgagtctatctctgggattccttccaggtttagtggcagcggatctgggacagattttactctttccatcaacagtgtggagtctgaagatatggcagattattactgtcaacaaaataataactggccgctcacgttcggtgctgggaccaagctggaactgaaa

SEQ ID NO: 3 - DNA, 408 bp, mus Musculus
atggaatggccttgtatctttctcttcctcctgtcagtaactgaaggtgtccactcccaggttcaccttcagcagtctggggctgagctggtgaggcctgggtcctcagtgaagatttcctgtaaggcttctggctatgaattcaatagtttctggatgaactgggtgaagcagaggcctggacagggtcttgagtggattggacagatttatcctggagatggtgatactaactacaatggaaaattcaagggtaaagccacactgactgctgacaaatcctccagcacagcctacatgcagctcagcagcctaacatctgaggactctgggatttacttctgtgcaagaggatacaaggcctggtttatttactggggccaagggactctggtcactgtctctgaa

SEQ ID NO: 4 - DNA, 381 bp, mus musculus
atggtatccacacctcagttccttgtatttttgcttttctggattccagcctccagaggtgacgtcttgctgactcagtctccagccattctgtctgtgagtccaggagaaagagtcagtttctcctgcagggccagtcagaacattggcacaagcatacactggtatcagcaaagcacaaatggttctccaaggcttatcataaagtatgcttctgagtctctctctgggatcccttccaggtttagtggcagtggatcagggacagattttactcttaccatcaacagtgtggagtctgaggatattgcagattattactgtcaacaaagtaatggctggccgctcacgttcggtggtgggaccaagctggagctgaaa

SEQ ID NO: 5 - DNA, 405 bp, mus Musculus
atgggatggagctggatctttctcttcctcctgtcaggaactgcaggtgtcctctctgaggtccagctgcaacagtctggacctgaactggtgaagcctaaaacttcaatgaagatatcctgcaaggcctctggttactcattcactgacttcaccatgaactgggtgaagcagagccatggaaaaaaccctgagtggattggacttattactccttacaatggtggaactagttacaaccagaagttcaagggcaaggccacatttactgtagacaggtcatccagcactgcctacatggaactcctcagtctgacatctgaggactctgcggtctattactgtgcaagaggcctgacctattttgaccagtggggccaaggcaccactctcacagtctcctca

SEQ ID NO: 6 - DNA, 387 bp, mus Musculus
atggattttcaagtgcagattttcagcttcctgctaatgagtgcctcagtcataatgtccaggggacaaattgttctcacccagtctccagcactcatgtctgcatctccaggggagaaggtcaccatgacctgcagtgccagctcaagtgtaagttacatgtactggtatcagcagaagccaacatcctcccccaaaccctggattttgctcacttccaacctggcttctggagtccctactcgcttcagtggcagtgggtctgggacctcttactctctcacaatcagcagcatggaggctgaagatgctgccacttattactgccagcagtggaatagtaaaccacccatcacgttcggaggggggaccaagctggaaataaaa

SEQ ID NO: 7 - DNA, 405 bp, mus Musculus; identical to SEQ ID NO: 5

SEQ ID NO: 8 - DNA, 387 bp, mus Musculus; identical to SEQ ID NO: 6

SEQ ID NO: 9 - DNA, 411 bp, mus Musculus
atggctgtcctggggctgcttctctgcctggtgacgttcccaagctgtgtcctgtcccaggtgcagctgaaggaatcaggacctggcctagtggcgccctcacagaacctgtccatcacatgcactgtctcaggtttctcattaaccgactatggtgtaaactgggttcgccagccttcaggaaagggtctggagtggctgggagaaatatgggctggtggaactacattctataattcagctctcaaatccagactgaccatcaccaaggacaactccaagagccaagttttcttagaaatgaacagtctgcaaagtcatgacacagccatgtactattgtgccaaacggcttaactgggacagttctatggactactggggtcaaggaacctcagtcaccgtctcctca

SEQ ID NO: 10 - DNA, 393 bp, mus Musculus
atggagacagacacactcctgttatgggtactgctgctctgggttccaggttccactggtgacattgtgctgacacagtctcctgcttcctttgctgtatctctgggacagagggccaccatctcatgcagggccagcgaaagtgtcagtacgtctgcctataattttctgcactggtaccagcagaaacctggacagccacccaaactcctcatctatcttgcatccaacctagaatctggggtccctgccaggttcagtggcagtgggtctgggacagacttcaccctcaacatccatcctgtggaggaggaggatgctgcaacctattactgtcagcacagtagggagcttccgtacacgttcggaggggggaccaagttggaaataaaa

SEQ ID NO: 11 - DNA, 405 bp, mus Musculus
atgagagtgctgattcttttgtggctgttcacagcctttcctggtatcctgtctgatgtgcagcttcaggagtcgggacctggcctggtgaaaccttctcagtctctgtccctcacctgcactgtcactggctactcaatcaccagtgattatgcctggaactggatccggcactttccaggaaacaaactggagtggatgggctacataagctacagtggtagcactagctacaacccatctctcaaaagtcgaatctctatcactcgagacacatccaagaaccagttcttcctgcagttgaattctgtgactactgaggacacagccacatattactgtgcaagagatggttactacacctttgctttctggggccaagggactctggtcactgtctctgca

SEQ ID NO: 12 - DNA, 393 bp, mus Musculus
atgaagttgcctgttaggctgttggtgctgatgttctggattcctgcttccagcagtgatgttgtgatgacccaaactccactctccctgcctgtcagtcttggagatcaagcctccatctcttgcagatctagtcagagccttgtacacagtaatggaaacacctatttacattggtacctgcagaagccaggccagtctccaaagctcctgatctacaaagtttccaaccgattttctggggtcccagacaggttcagtggcagtggatcagggacagatttcacactcaagatcagcagagtggaggctgaggatctgggagtttatttctgctctcaaagtacacatgttccgtacacgttcggaggggggaccaagctggaaataaaa

SEQ ID NO: 13 - protein, 140 aa, mus Musculus
MRVLILLCLFTAFPGVLSDVQVQESGPDLVKPSQSLSLTCTVTGHSITRGSSWHWIRQFPGNKLEWMGYIHYGGGTSYNPSLKSRISITRDTSKNQFFLQLNSVTTEDTATFFCARYSYDITYRWFFDVWGAGTTVIVSS

SEQ ID NO: 14 - protein, 127 aa, mus Musculus
MVSTPQFLVFLLFWIPASRGDILLTQSPAILSVSPGERVSFSCRASQNIGTSIHWYQQRKNGSPRLLIKYASESISGIPSRFSGSGSGTDFTLSINSVESEDMADYYCQQNNNWPLTFGAGTKLELK

SEQ ID NO: 15 - protein, 136 aa, mus Musculus
MEWPCIFLFLLSVTEGVHSQVHLQQSGAELVRPGSSVKISCKASGYEFNSFWMNWVKQRPGQGLEWIGQIYPGDGDTNYNGKFKGKATLTADKSSSTAYMQLSSLTSEDSGIYFCARGYKAWFIYWGQGTLVTVSE

SEQ ID NO: 16 - protein, 127 aa, mus Musculus
MVSTPQFLVFLLFWIPASRGDVLLTQSPAILSVSPGERVSFSCRASQNIGTSIHWYQQSTNGSPRLIIKYASESLSGIPSRFSGSGSGTDFTLTINSVESEDIADYYCQQSNGWPLTFGGGTKLELK

SEQ ID NO: 17 - protein, 135 aa, mus Musculus
MGWSWIFLFLLSGTAGVLSEVQLQQSGPELVKPKTSMKISCKASGYSFTDFTMNWVKQSHGKNPEWIGLITPYNGGTSYNQKFKGKATFTVDRSSSTAYMELLSLTSEDSAVYYCARGLTYFDQWGQGTTLTVSS

SEQ ID NO: 18 - protein, 129 aa, mus musculus
MDFQVQIFSFLLMSASVIMSRGQIVLTQSPALMSASPGEKVTMTCSASSSVSYMYWYQQKPTSSPKPWILLTSNLASGVPTRFSGSGSGTSYSLTISSMEAEDAATYYCQQWNSKPPITFGGGTKLEIK

SEQ ID NO: 19 - protein, 135 aa, mus Musculus; identical to SEQ ID NO: 17

SEQ ID NO: 20 - protein, 129 aa, mus Musculus; identical to SEQ ID NO: 18

SEQ ID NO: 21 - protein, 137 aa, mus Musculus
MAVLGLLLCLVTFPSCVLSQVQLKESGPGLVAPSQNLSITCTVSGFSLTDYGVNWVRQPSGKGLEWLGEIWAGGTTFYNSALKSRLTITKDNSKSQVFLEMNSLQSHDTAMYYCAKRLNWDSSMDYWGQGTSVTVSS

SEQ ID NO: 22 - protein, 131 aa, mus Musculus
METDTLLLWVLLLWVPGSTGDIVLTQSPASFAVSLGQRATISCRASESVSTSAYNFLHWYQQKPGQPPKLLIYLASNLESGVPARFSGSGSGTDFTLNIHPVEEEDAATYYCQHSRELPYTFGGGTKLEIK

SEQ ID NO: 23 - protein, 135 aa, mus Musculus
MRVLILLWLFTAFPGILSDVQLQESGPGLVKPSQSLSLTCTVTGYSITSDYAWNWIRHFPGNKLEWMGYISYSGSTSYNPSLKSRISITRDTSKNQFFLQLNSVTTEDTATYYCARDGYYTFAFWGQGTLVTVSA

SEQ ID NO: 24 - protein, 131 aa, mus Musculus
MKLPVRLLVLMFWIPASSSDVVMTQTPLSLPVSLGDQASISCRSSQSLVHSNGNTYLHWYLQKPGQSPKLLIYKVSNRFSGVPDRFSGSGSGTDFTLKISRVEAEDLGVYFCSQSTHVPYTFGGGTKLEIK

SEQ ID NO: 25 - protein, 6 aa, mus Musculus
RGSSWH

SEQ ID NO: 26 - protein, 16 aa, mus Musculus
YIHYGGGTSYNPSLKS

SEQ ID NO: 27 - protein, 13 aa, mus Musculus
YSYDITYRWFFDV

SEQ ID NO: 28 - protein, 11 aa, mus Musculus
RASQNIGTSIH

SEQ ID NO: 29 - protein, 7 aa, mus Musculus
YASESIS

SEQ ID NO: 30 - protein, 9 aa, mus Musculus
QQNNNWPLT

SEQ ID NO: 31 - protein, 5 aa, mus Musculus
SFWMN

SEQ ID NO: 32 - protein, 17 aa, mus Musculus
QIYPGDGDTNYNGKFKG

SEQ ID NO: 33 - protein, 8 aa, mus Musculus
GYKAWFIY

SEQ ID NO: 34 - protein, 11 aa, mus Musculus
RASQNIGTSIH

SEQ ID NO: 35 - protein, 7 aa, mus Musculus
YASESLS

SEQ ID NO: 36 - protein, 9 aa, mus Musculus
QQSNGWPLT

SEQ ID NO: 37 - protein, 5 aa, mus Musculus
DFTMN

SEQ ID NO: 38 - protein, 17 aa, mus Musculus
LITPYNGGTSYNQKFKG

SEQ ID NO: 39 - protein, 7 aa, mus Musculus
GLTYFDQ

SEQ ID NO: 40 - protein, 10 aa, mus Musculus
SASSSVSYMY

SEQ ID NO: 41 - protein, 7 aa, mus Musculus
LTSNLAS

SEQ ID NO: 42 - protein, 10 aa, mus musculus
QQWNSKPPIT

SEQ ID NO: 43 - protein, 5 aa, mus Musculus
DFTMN

SEQ ID NO: 44 - protein, 17 aa, mus Musculus
LITPYNGGTSYNQKFKG

SEQ ID NO: 45 - protein, 7 aa, mus Musculus
GLTYFDQ

SEQ ID NO: 46 - protein, 10 aa, mus musculus
SASSSVSYMY

SEQ ID NO: 47 - protein, 7 aa, mus Musculus
LTSNLAS

SEQ ID NO: 48 - protein, 10 aa, mus Musculus
QQWNSKPPIT

SEQ ID NO: 49 - protein, 5 aa, mus Musculus
DYGVN

SEQ ID NO: 50 - protein, 16 aa, mus musculus
EIWAGGTTFYNSALKS

SEQ ID NO: 51 - protein, 10 aa, mus Musculus
RLNWDSSMDY

SEQ ID NO: 52 - protein, 15 aa, mus musculus
RASESVSTSAYNFLH

SEQ ID NO: 53 - protein, 7 aa, mus Musculus
LASNLES

SEQ ID NO: 54 - protein, 9 aa, mus musculus
QHSRELPYT

SEQ ID NO: 55 - protein, 6 aa, mus Musculus
SDYAWN

SEQ ID NO: 56 - protein, 16 aa, mus musculus
YISYSGSTSYNPSLKS

SEQ ID NO: 57 - protein, 8 aa, mus Musculus
DGYYTFAF

SEQ ID NO: 58 - protein, 16 aa, mus Musculus
RSSQSLVHSNGNTYLH

SEQ ID NO: 59 - protein, 7 aa, mus musculus
KVSNRFS

SEQ ID NO: 60 - protein, 9 aa, mus musculus
SQSTHVPYT